European Patent Specification EP 4 430 401 B1, published April 30, 2025. Title: Collagen Type XXII Assay. Applicant: Nordic Bioscience A/S. The sequence listing filed with the application follows.

SEQUENCE LISTING (22 sequences)

SEQ ID NO: 1 - protein, 10 aa, Homo sapiens
AARPGNVKGP

SEQ ID NO: 2 - protein, 11 aa, synthetic construct
  VARIANT 11: note = wherein X is any amino acid
AARPGNVKGPX

SEQ ID NO: 3 - protein, 11 aa, Homo sapiens
AARPGNVKGPA

SEQ ID NO: 4 - protein, 9 aa, Homo sapiens
AARPGNVKG

SEQ ID NO: 5 - protein, 11 aa, Mus musculus
KASQDIYSSLS

SEQ ID NO: 6 - protein, 7 aa, Mus musculus
RANRLIN

SEQ ID NO: 7 - protein, 9 aa, Mus musculus
LQYDDFPYM

SEQ ID NO: 8 - protein, 5 aa, Mus musculus
TYGVH

SEQ ID NO: 9 - protein, 16 aa, Mus musculus
AIWRGGSTDYNPAFMS

SEQ ID NO: 10 - protein, 9 aa, Mus musculus
RSTLFYFDY

SEQ ID NO: 11 - protein, 74 aa, Mus musculus
KASQDIYSSLSWFQQKPGKSPKTLIYRANRLINGVPSRFSGSGSGQDYSLTISSLEYEDVGIYYCLQYDDFPYM

SEQ ID NO: 12 - protein, 76 aa, Mus musculus
TYGVHWIRQSPGKGLEWLGAIWRGGSTDYNPAFMSRLSITKDISKSQVFFKMNSLQADDTAIYYCAKRSTLFYFDY

SEQ ID NO: 13 - protein, 107 aa, Mus musculus
DIKMTQSPSSMHASLGERVTITCKASQDIYSSLSWFQQKPGKSPKTLIYRANRLINGVPSRFSGSGSGQDYSLTISSLEYEDVGIYYCLQYDDFPYMFGGGTKLEIK

SEQ ID NO: 14 - protein, 116 aa, Mus musculus
QVQLKQSGPSLVQPSQSLSITCTVSGFSLTTYGVHWIRQSPGKGLEWLGAIWRGGSTDYNPAFMSRLSITKDISKSQVFFKMNSLQADDTAIYYCAKRSTLFYFDYWGQGTTLTVS

SEQ ID NO: 15 - protein, 10 aa, synthetic construct
  MOD_RES 1: note = Amino acid is biotinylated via an optional linker
AARPGNVKGP

SEQ ID NO: 16 - protein, 30 aa, Homo sapiens
GPPGPPGQCDPSQCAYFASLAARPGNVKGP

SEQ ID NO: 17 - protein, 30 aa, synthetic construct
PGMRGMPGSPGGPGSDGKPGPPGSQGESGR

SEQ ID NO: 18 - protein, 10 aa, synthetic construct
  MOD_RES 10: note = Amino acid is biotinylated
PPGSQGESGR

SEQ ID NO: 19 - protein, 13 aa, synthetic construct
  MOD_RES 1: note = Amino acid is bound to keyhole limpet hemocyanin
CGGAARPGNVKGP

SEQ ID NO: 20 - protein, 257 aa, Mus musculus
QVQLKQSGPSLVQPSQSLSITCTVSGFSLTTYGVHWIRQSPGKGLEWLGAIWRGGSTDYNPAFMSRLSITKDISKSQVFFKMNSLQADDTAIYYCAKRSTLFYFDYWGQGTTLTVSSAKTTPPSVYPLAPGCGDTTGSSVTLGCLVKGYFPESVTVTWNSGSLSSSVHTFPALLQSGLYTMSSSVTVPSSTGQVRPSPAALLTQPAAPRWTKNLSPAGPFQQSTPVLHARSVTNAQLLTSRVDHPSSSSLQISRMYS

SEQ ID NO: 21 - protein, 214 aa, Mus musculus
DIKMTQSPSSMHASLGERVTITCKASQDIYSSLSWFQQKPGKSPKTLIYRANRLINGVPSRFSGSGSGQDYSLTISSLEYEDVGIYYCLQYDDFPYMFGGGTKLEIKRADAAPTVSIFPPSSEQLTSGGASVVCFLNNFYPKDINVKWKIDGSERQNGVLNSWTDQDSKDSTYSMSSTLTLTKDEYERHNSYTCEATHKTSTSPIVKSFNRNEC

SEQ ID NO: 22 - protein, 10 aa, synthetic construct
  MOD_RES 10: note = Amino acid is biotinylated
PGMRGMPGSP